European Patent Application EP 4 755 897 A1, published June 10, 2026. Title: METHOD FOR PRODUCING OLIGONUCLEOTIDE. Applicant: NIPPON SHOKUBAI CO., LTD. Application EP 24849236.5, filed August 1, 2023. The sequence listing filed with the application follows.

SEQUENCE LISTING (3 sequences)

SEQ ID NO: 1 - RNA, 21 nt, synthetic construct
  source 1..21: mol_type = other RNA
actgttatactcagaatcgcg

SEQ ID NO: 2 - RNA, 21 nt, synthetic construct
  source 1..21: mol_type = other RNA
  modified_base order(2,4,11,16): mod_base = OTHER; note = 2-prime-O-fluoro RNA nucleotides
  modified_base order(6,9,14,20): mod_base = OTHER; note = 2-prime-O-methyl RNA nucleotides
actgttatactcagaatcgcg

SEQ ID NO: 3 - DNA, 22 bp, synthetic construct
  source 1..22: mol_type = other DNA
  modified_base 1^2: mod_base = OTHER; note = residues linked by phosphorothioate internucleotide linkage
  modified_base order(2,8): mod_base = OTHER; note = 2-prime-O,4-prime-C-methylene bridged nucleotides
  modified_base order(5,15,20,22): mod_base = OTHER; note = 2-prime-O-methyl RNA nucleotides
  modified_base order(14,16,17): mod_base = OTHER; note = 2-prime-O-methoxyethyl RNA nucleotides
  modified_base order(3,4,6,7,9,11,12,13,18,19,21): mod_base = OTHER; note = 2-prime-fluoro RNA nucleotides
  modified_base order(4,6,7,9,11,18): mod_base = OTHER; note = uracil
gactgttatactcagaatcgcg